European Patent Specification EP 3 801 507 B1, published January 1, 2025. Title: TOMM6-interacting extracts and compounds for use in the treatment and prophylaxis of nervous system diseases. Applicant: ETH Zurich. The sequence listing filed with the application follows.

SEQUENCE LISTING (18 sequences)

SEQ ID NO: 1 - protein, 74 aa, Homo sapiens
MASSTVPVSAAGSANETPEIPDNVGDWLRGVYRFATDRNDFRRNLILNLGLFAAGVWLARNLSDIDLMAPQPGV

SEQ ID NO: 2 - protein, 74 aa, Mus musculus
MASSGVTVSAAGSASEASEVPDNVGDWLRGVFRFATDRNDFRRNLILNLGLFAAGVWLARNLSDIDLMAPQPGV

SEQ ID NO: 3 - protein, 63 aa, Danio rerio
MSGKKSEGKSGGVTGWISSACRFAADRNDFRRNLLVNLGLFAAGVWVARNLSDFDLMSPQPVT

SEQ ID NO: 4 - protein, 74 aa, Mus musculus; identical to SEQ ID NO: 2

SEQ ID NO: 5 - protein, 14 aa, Mus musculus
NLSDIDLMAPQPGV

SEQ ID NO: 6 - protein, 14 aa, Artificial Sequence
  Partial peptide sequence of mouse TOMM6 with oxidized M
  MISC_FEATURE (8)..(8): oxidized
NLSDIDLMAPQPGV

SEQ ID NO: 7 - protein, 15 aa, Artificial Sequence
  Partial peptide sequence of mouse TOMM6 with oxidized M
  MISC_FEATURE (9)..(9): oxidized
RNLSDIDLMAPQPGV

SEQ ID NO: 8 - DNA, 348 bp, Artificial Sequence
  Partial sequence of vector pcDNA3.1 carrying the human TOMM6 gene
ccactagtaacggccgccagtgtgctggaattcatggcttccagcactgtcccggtgagcgctgctggctcggctaatgaaactcccgaaataccggacaacgtgggagattggcttcggggcgtctaccgctttgccactgataggaatgacttccggaggaacttgatactaaatttgggactctttgctgcgggagtttggctggccaggaacttgagtgacattgacctcatggcacctcagccaggggtgtagctcgagcatgcatctagagggccctattctatagtgtcacctaaatgctagagctcgctgatcagcctcgactgtgccttctagttgcca

SEQ ID NO: 9 - DNA, 34 bp, Artificial Sequence
  primer TOMM6 forward
tatttagaattcatggcttccagcactgtcccgg

SEQ ID NO: 10 - DNA, 34 bp, Artificial Sequence
  primer TOMM6 reverse
tatttactcgagctacacccctggctgaggtgcc

SEQ ID NO: 11 - DNA, 30 bp, Artificial Sequence
  primer TOMM6-internal forward
ggtgagcgctgctggctcggctaatgaaac

SEQ ID NO: 12 - DNA, 30 bp, Artificial Sequence
  primer pcDNA3-reverse
tagaaggcacagtcgaggctgatcagcgag

SEQ ID NO: 13 - DNA, 429 bp, Artificial Sequence
  Partial sequence of vector CosSHa.Tet carrying the human TOMM6 gene
gtcacacatttgttctgcaacagatgtcaagtgcttcagcctgcgtgctggacaatgacgtgttgctggagtacaatgatgccttgttcttcattttgcagatcagtcgacaccatggcttccagcactgtcccggtgagcgctgctggctcggctaatgaaactcccgaaataccggacaacgtgggagattggcttcggggcgtctaccgctttgccactgataggaatgacttccggaggaacttgatactaaatttgggactctttgctgcgggagtttggctggccaggaacttgagtgacattgacctcatggcacctcagccaggggtgtaggtcgacctccctgcttgtacttcctcgttcttgtggtctaggctgggggaggggttatccaccgtagctcttttaattgaggtggtggct

SEQ ID NO: 14 - DNA, 30 bp, Artificial Sequence
  primer CosSHa.Tet-forward
gcttcagcctgcgtgctggacaatgacgtg

SEQ ID NO: 15 - DNA, 31 bp, Artificial Sequence
  primer TOMM6-reverse
cctggctgaggtgccatgaggtcaatgtcac

SEQ ID NO: 16 - DNA, 28 bp, Artificial Sequence
  primer Prp-forward
aagcggccaaagcctggagggtggaaca

SEQ ID NO: 17 - DNA, 25 bp, Artificial Sequence
  primer APP-forward
ctgaccactcgaccaggttctgggt

SEQ ID NO: 18 - DNA, 29 bp, Artificial Sequence
  primer Prp-reverse
gtggataacccctcccccagcctagacca